European Patent Application EP 4 600 259 A1, published August 13, 2025. Title: KERATIN YK93-8, AND PREPARATION METHOD THEREFOR, PHARMACEUTICAL COMPOSITION THEREOF AND USE THEREOF. Applicant: Institute of Materia Medica Chinese Academy Of Medical Sciences. The sequence listing filed with the application follows.

SEQUENCE LISTING (2 sequences)

SEQ ID NO: 1 - protein, 591 aa, Manis pentadactyla
MSCRSYRVSSGRQIGNFSSCSAVMPQSLSRFRASSVSCRSGPGFRGLGGFGSRSVIAFGSCPPRMAAVGPRPIRCGVGFSAGSGLAFGLGDSCGAGLGFGTGSGLGYGFGGPGFGYRIGGVGVPAAPSITAVTVNQSLLTPLNLEIDPNAQRVKRDEKEQIKTLNNKFASFIDKVRFLEQQNKLLETKWNFLQDQKGVQSNLEPLFENYVANLRRQLDIVSSDQARLETERNNMQDVLEGFKKKYEEEVVFRANAENEFVALKKDVDAAFLNKSDLEANVDALIQEIDFLKNLYMAEIQLLQSHISDTSVIVKMDNSRDLNFDGIIAEVKAQYEEVARRSRADAEAWYQTKYEEMRMTAGQHSDNLRNTRDEINELTRVIQRLKAEIEHTKAQRAKLEAAIAEAEQQGEAALNDAKCKLADLEAALQQAKQDMARQLREYQELMNIKLALDIEIATYRRLLEGEEIRICEGVGPVNISVSSSRGGVVCGPEPLLTSSTLSRGGVTFSGGSSIRSSGACGLSLGGSRVVAAGGDVLSAGSRGGSVLVGDACAPSIPCPLPTDGGFSSCSGGRSSLGSSVRFVSTTTSRRTKY

SEQ ID NO: 2 - DNA, 1773 bp, Manis pentadactyla
  source 1..1773: mol_type = genomic DNA
atgagttgtcgtagctatcgcgtgagcagtggtcgccagattggcaattttagtagctgtagtgccgtgatgccgcagagcctgagtcgctttcgtgccagtagtgtgagctgccgcagtggtccgggttttcgtggcctgggtggttttggcagccgcagtgttattgcctttggtagctgcccgccgcgcatggccgcagttggtcctcgtccgattcgctgcggcgtgggctttagcgcaggtagcggtctggcctttggtctgggcgatagctgtggtgccggtctgggctttggcaccggcagtggtctgggttatggttttggcggtccgggctttggctatcgtattggcggcgttggcgttccggcagcaccgagtattaccgcagttaccgtgaatcagagtctgctgaccccgctgaatctggaaattgatccgaatgcccagcgtgtgaaacgcgatgaaaaagaacagattaagaccctgaataataagtttgccagctttattgataaggttcgctttctggaacagcagaataagctgctggaaaccaaatggaattttctgcaggatcagaaaggtgtgcagagcaatctggaaccgctgtttgaaaattatgtggccaatctgcgtcgccagctggatattgtgagcagcgatcaggcacgcctggaaaccgaacgtaataatatgcaggatgtgctggaaggctttaaaaagaaatatgaagaagaggttgtgttccgtgcaaatgccgaaaatgaatttgtggccctgaaaaaagatgttgatgcagcctttctgaataagagcgatctggaagccaatgtggatgcactgattcaggaaattgattttctgaaaaacctgtatatggccgaaattcagctgctgcagagccatattagtgataccagcgttattgtgaaaatggataatagtcgtgatctgaatttcgatggtattattgccgaagtgaaagcccagtatgaagaagttgcccgccgcagtcgcgcagatgcagaagcctggtatcagaccaaatatgaagagatgcgtatgaccgccggtcagcatagtgataatctgcgtaatacccgcgatgaaattaatgaactgacccgtgtgattcagcgcctgaaagcagaaattgaacataccaaagcacagcgtgccaaactggaagccgcaattgcagaagccgaacagcagggcgaagcagcactgaatgatgccaaatgcaaactggcagatctggaagcagccctgcagcaggcaaaacaggatatggcccgtcagctgcgcgaatatcaggaactgatgaatattaagctggcactggatattgaaattgccacctatcgtcgcctgctggaaggcgaagaaattcgtatttgcgaaggtgttggcccggtgaatattagcgtgagtagcagccgtggcggtgtggtgtgcggccctgaaccgctgctgaccagtagtaccctgagccgtggcggcgttacctttagtggcggcagtagcattcgcagcagcggcgcctgtggcctgagcttaggcggcagtcgtgttgttgcagccggtggtgacgttctgagtgcaggtagtcgcggtggtagcgttctggtgggcgatgcctgtgcaccgagcattccgtgcccgctgccgaccgatggcggctttagcagctgtagtggcggtcgtagcagcctgggtagcagtgttcgctttgtgagcaccaccaccagtcgtcgcaccaaatat